European Patent Application EP 4 782 543 A1, published July 29, 2026. Title: 一种低氧特异性基因表达盒、包含其的细菌及应用. Applicant: 上海缮维特生物技术有限公司. The sequence listing filed with the application follows.

SEQUENCE LISTING (146 sequences)

SEQ ID NO: 1 - DNA, 237 bp, Artificial sequence
  source 1..237: mol_type = other DNA
gcgtgaacgcagtttatctaacacgagctttactccctgtttcaatagtcctgttattttgccatatccaataaatcacatggcggcgtaaatcaacaattgggtctgattttctaccccattattggtgttaccaatacgcctttaactgccttaaatcaaaaattgtcgcagcaaggttaactaaaatccctgttcgttaacaattttgcgtctcagacgtaaccctcaggataa

SEQ ID NO: 2 - DNA, 185 bp, Artificial sequence
  source 1..185: mol_type = other DNA
cgctgcactggtaaaagacgcgatgtataacggttctttgttgattcgtctgttgcagggttaacattttttaactgttctaccaaaatttgcgctatctcaatttgggccaggaaagcataacttagactttcaaggttaattattttcctggtttatatttgtgaagcataacggtggagtta

SEQ ID NO: 3 - DNA, 1167 bp, Artificial sequence
  source 1..1167: mol_type = other DNA
ctcttcataaaacccgtcagtgtaagctggcgggtttttgcttttaccgggcgacaggatgaatgactgtccacgacgctatacccaaaagaaagcggcttatcggtcagtatcatctcttcataaaacccgtcagtgtaagctggcgggtttttgcttttacagggcggcaggatgaatgactgtccacgacgctatacccgaaagaaagcggcttatcggtcagtttcacctcttcataaaacccgtcagtgtaagctggcgggtttttgcttttacagggcggcaggatgaatgactgtccacgacgctatacccgaaagaaagcggcttatcggtcagtttcatctcttcataaaccccgtcagtgtaagctggcgggtttttgcttttacagggcgacaggatgaatgactgtccacgacgctatacccgaaagaaagcggcttatcggtcagtttcacctcttcataaaatccgcttcggcgggtttttgcttatcaggccggtgaagggtatagaggttgcagaagacgccagcgtcaccatccggcaattaattgacagccgtggtgacataatattattcgtttttgtgatgagaaacacaaaacgctatgtattgcgctatttttagttgaagtgaaaagcaatcgatttctttcacaaaattacatcctgaaaaacagcaagaaagcggtgtaaattatttgttttaaatgaaaattaaatgtatgaaatattttggttaaaattttattaaatgtttctttgcaaacaaataaggtaaaaaaatgtgacgcgtaacggtttttaagcgcatttaccttcggtttatacttaaatttgagaaattacgttttaaatttaacgctggaattgtcgataaaatgtcccgtaattgattgaaatatcgtcttcatgggatatcaaaaataggagataaaataggctggttatcgccataatatatcgttatcccgcccctgttttttgattgaaatcaggctaagttactgctttatttttgtaacctattgaaatatcaggttttctttatttaataaaaaccatgtaaaaattgtggtaagttaatttgtgagtggtcgcacataacctttaagatttaatttgctacacttcctgccgttcacaatgttatttcag

SEQ ID NO: 4 - DNA, 317 bp, Artificial sequence
  source 1..317: mol_type = other DNA
gctcattaaatttaactcaaattttgcctggtaattatccggtaattgcttgaaatatggtctcagccccttttttgtattaaccacataacgaatgatgttatcgccataaaatatggttatccccgtcattttttttgacaaaaatcagggtttatgctgatttttatactttaacttgttgatatttaaaggtatttaattgtaataacgatactctggaaagtattgaaagttaatttgtgagtggtcgcacatatcctgttcatttcattttgatacacttcatgccgtcaatgaggtaattaacgtaggtc

SEQ ID NO: 5 - DNA, 295 bp, Artificial sequence
  source 1..295: mol_type = other DNA
cgtaacgctaaaaccaacaccggccgcagccagcggcattgccagcatgcctgcgccaattgtggttcccgccacgataaaaacacttcccagggttctgtttttcacgctttcttctgtcctgacgatctttatgagtgatatctgcggcgcaggttaaggcataacggctgcttcgtcaaaccgacgttacatatggtgtaaatataaatgtacaataaaaagcattcagtcctgcgctggcgcaaagtcttcataagcggcaatcgctacgctaggctttttttgaggaggg

SEQ ID NO: 6 - DNA, 174 bp, Artificial sequence
  source 1..174: mol_type = other DNA
agacgcgatgtataacggctctttgttgattcgtctattacagggttaacattttttaactgttgtacaaaaatttgcgctaactcaagctgattgcccttgccatatcttagactttctccactgtattattttcctggcttatattttcgaagcataacggtggagttagtg

SEQ ID NO: 7 - DNA, 574 bp, Artificial sequence
  source 1..574: mol_type = other DNA
gttaatattggcggggtggatttatgcctttattagtaatcctgaaactctgcgtcgtattagccagtgaccaaaaaaagaattaaggtcaaccgtgctgtttttgcttcgtctctttttatctttaattgccaaccgaaactaatttcagccttataactcacacattttaaacataaatgtcactaaagttaccttattgaaacatgattaacataatttgtaggaattgatatttatcaatgtataagtcttggaaatgggcatcaaaaagagataaattgttctcgatcaaattggctgaaaggcggtaatttagctataaattgatcaccgtcgaaaaatgcaaatttgcttcaacaaaaacctgtttattgtaaggattttgcggcgtaatatatacgtgggatcaatttgagtttttattaacatgtttgcaacctttctttacgccgtttttgtgtgcattcacatggtatgatgaaagtgttcaaacaaatttctattggggcatgcgtgtgaccctttctaacggggttcactctcggagtcttcatgcgatgagcaaggagtc

SEQ ID NO: 8 - DNA, 426 bp, Artificial sequence
  source 1..426: mol_type = other DNA
aaagcagcattctgggcaaaataaaatcaaatagcctacgcaatgtaggcttaatgattagtctgagttatattacggggcgtttttttaatgccccgctttacatatatttgcattaataaaataattgtaattataaggttaaatatcggtaatttgtatttaataaatacgatcgatattgttactttattcgcctgatgctcccttttaattaactgttttagcggaggatgcggaaaaaattcaactcatttgttaatttttaaaatttatttttatttggataatcaaatatttactccgtatttgcataaaaaccatgcgagttacgggcctataagccaggcgagatatgatctatatcaatttctcatctataatgctttgttagtatctcgtcgccgacttaataaagagagagtt

SEQ ID NO: 9 - DNA, 370 bp, Artificial sequence
  source 1..370: mol_type = other DNA
aacattatttgccgttgtaataacgacccggaattataacggctaaataaccatcaattgataaaaaatatatttgtctttttgtgcgcaacagaattttggaaattattggtaatttctacgctacctattttctttacacgattcagccgattaaatttaaatttctgccgttgattgtccttttattgataataaattgttaagtaattgttttatttttacattggttataccaattatccctcaacatcccacttacagacctcatccgttataacgcaaagtttcaacagtgtcttaaagttatttcgacatacttggcaacatatgtgacatgcgcggcagaacttggtaacacagaaccaat

SEQ ID NO: 10 - DNA, 826 bp, Artificial sequence
  source 1..826: mol_type = other DNA
ccgacatgtccgatagcattattgccatcggacatattttaccaggcggcgttatacgcccgcctggtcctctgataagtcccggaccgattgactgaagatgttcaggtaaatgaggacgcactctcaaactatttttagcccttgagcgccgttaacgcgggcgtaatacatctcgagtaatcactaactagccatatatgaaatcgcctgttaatggtaccaatagccttgacgcaatagagtaatgacaaaaattaaaacaagtcagcgttactggcgtaagtatgccgcataaaattttgcataaataatgccgttttagcgatgggagagaggacacgttaattattccattttaaccttatatatgttcaatattcaatgggttatggatgttttcagcattaatacccgcagtagctaatgattatcttttttagtctcctgccgatgaaataatcgtgtaatctttctgtaagagactgacaatgacgcaataatgtttggttaatgcttggtgaatatattgttgcattattgatgttttgtgttgtacttagtagtaatagcggtagttccccggcagtgatggtcactcactatggagatcgcgaatggtaatgtccgcaccaggacacattgtttacagtagttacaacaccctgtacggacattctctctccggtggtggtcttgtcatcttaaaagctctcatcatttcccttactgaccatacccatgacgtcatatgtggtgcgcgtagccgtgtgtggcgtcgtttcaaaaagcaagctaaggcttacaaggaagccaaccctcagat

SEQ ID NO: 11 - DNA, 298 bp, Artificial sequence
  source 1..298: mol_type = other DNA
tgaagtaacaacactcccgacatcaaaggcaatggcataatgccattgccttttcacttccctttgctgtcctctcccctcaattggccctaccaattttagccagttaccacagcctactcacatttcattaaattaactctacaataccgttgccaataaataacatctggttaactatttgttgtcattatccatacacaacaatattggcaggaccacttttacacataatgtgaccccaacgagatgagcaaagattcatcccattatgcgtgtggttctcaggagacctgca

SEQ ID NO: 12 - DNA, 291 bp, Artificial sequence
  source 1..291: mol_type = other DNA
tagcgttgtctgtttagcgtgcattattgtccctgttgccctgtttcagggcaattttgtaaccgcgatcatatcctcaacatttaattcgttaaaagccgccgaaacgctgcggttcaaccgtcatacctgctatcttcaacatcaggacaatattgcaacgttttattaacaaatttaacgtcgaatcgttttgctgacgtgaaaatggcataagacctgcatgaaaaagtctgcaaacacacaacgccacgtaaaacataagaaaatgacgccacttgaggggtatgt

SEQ ID NO: 13 - DNA, 292 bp, Artificial sequence
  source 1..292: mol_type = other DNA
aatgtcatgcctccagtgaatgttacctggagtgtagaaaacctcatccattccggggagaagaatttataaagtgtgatccgacctgaattcattatgcagaacggattgacatgagctggcatatccccgaccagatcgcggcttaacacgcttaacggcagttgaatcatcagtaaaataaaacagttgtaacttgaaatggtaaaatgttaataatattttgctatcaggttatcaaaaacaaacaactttacttgtcacccgcacggctctgtttttaacatcgctt

SEQ ID NO: 14 - DNA, 344 bp, Artificial sequence
  source 1..344: mol_type = other DNA
tgtttttaggcggataaggcatttgtgcgcagatgcctgatgcgacgcttgcgcgtcttatcatgcctacaatcagtgcgggtttggtaggctggataaggcgttcacgccgcatccggcgatcgtgcactgatgcctgatgcaaatcctgctgaaagcacacagcttttttcatcactgtcatcactctgtcatctttccagtagaaactaatgtcactgaaatggtgttttatagttaaatataagtaaatatattgttgcaataaatgcgagatctgttgtacttattaagtagcagcggaagttcccggcagtgatagtcagtcactatggagatcgcgg

SEQ ID NO: 15 - DNA, 371 bp, Artificial sequence
  source 1..371: mol_type = other DNA
gaacacagtatctacagggtgattctgcacattcctataggccgagtaaggtgttcacgccgcatccggcaagataaggcgctctggatcaacaacctaagggcaattctctgatgaggattgcccttttctttaccagacatctccccccacaagaattggccctaccaattcttcgcttatctgacctctggttcacaatttcccaattaaaactcacatcaatgttgccaatacataacatttagttaaccattcattgtcattatccctacacaacacaattggcagtgccacttttacacaacgtgtgacaaggagatgagcaacagactcattacacgatgtgcgtggactccaggagacctgca

SEQ ID NO: 16 - DNA, 274 bp, Artificial sequence
  source 1..274: mol_type = other DNA
ctgacattgcctgcgaaaactgttcccgaatctcatccgccgtgatgctgttcgccatagtgtctgcctccagtggtcagtaatctggagtgtaggtaaccgcattcactcttgcgggaagaatttacaaactgtgatctcgccgcgaaaacatcaatattatccattttgctgtaacataattgctttaattgttaataatattttgcaatcaagttatcataatcaaacaacttcacttgtcagcgacaccgcttcgtttttaacatcgctt

SEQ ID NO: 17 - DNA, 1080 bp, Artificial sequence
  source 1..1080: mol_type = other DNA
atgcaagcggcaacagtcgtcattaaccgccgcgctctgcgacacaacctgcaacgtctgcgtgaactggcgcctgccagtaagctggttgcggtggtgaaagcgaacgcttatggacacggtcttctggagaccgcgcgaacgctccctgatgctgacgcttttggcgtggcgcgtcttgaagaggctctacgtctgcgagcgggcgggatcacgcagccaatcctgctgctggagggttttttcgacgccgccgatttgccgaccatttccgcgcaatgtctgcataccgccgtacataatcaagagcagcttgccgccctggaggcggtggagctggcggagccggtaacggtctggatgaagctggataccggtatgcatcgtctcggcgtgcgtcccgaagaggcggaggcgttctaccagcgtctgacgcactgtaaaaatgtacgccagccggtgaatatcgtcagccattttgcccgtgcggatgagccggaatgcggcgctaccgaacatcagctcgacatttttaatgccttctgtcagggtaaacccggtcagcgctctattgccgcgtctggcggtatcctgctgtggccgcagtctcactttgactgggcgcgtccgggcatcattttgtatggcgtatcgccgctggagcacaaaccctgggggccggattttggttttcagccggtgatgtccttaacctccagtttgatcgcggtgcgtgaccacaaagcgggcgaaccggtgggctacggcgggacatgggtgagtgagcgcgacacgcgcctgggcgtggtggcgatgggttatggcgatggctacccacgagcggcgccttccggtacgccagtactggtcaatggtcgtgaagttccgattgtcgggcgggtggcgatggatatgatttgcgtagatttggggccaaacgcgcaggataacgcgggcgatccggtggtcttatggggtgaaggtctgccggttgaacgtatcgctgaaatgacaaaagtaagtgcttacgaacttatcacgcgcctgacctcaagggtggcgatgaagtatattgattaa

SEQ ID NO: 18 - protein, 359 aa, Artificial sequence
MQAATVVINRRALRHNLQRLRELAPASKLVAVVKANAYGHGLLETARTLPDADAFGVARLEEALRLRAGGITQPILLLEGFFDAADLPTISAQCLHTAVHNQEQLAALEAVELAEPVTVWMKLDTGMHRLGVRPEEAEAFYQRLTHCKNVRQPVNIVSHFARADEPECGATEHQLDIFNAFCQGKPGQRSIAASGGILLWPQSHFDWARPGIILYGVSPLEHKPWGPDFGFQPVMSLTSSLIAVRDHKAGEPVGYGGTWVSERDTRLGVVAMGYGDGYPRAAPSGTPVLVNGREVPIVGRVAMDMICVDLGPNAQDNAGDPVVLWGEGLPVERIAEMTKVSAYELITRLTSRVAMKYID

SEQ ID NO: 19 - DNA, 1071 bp, Artificial sequence
  source 1..1071: mol_type = other DNA
atgacccgccctatacaggccagccttgatttacaggtaatgaaacaaaatttggctattgtgcgccgggcggccccagaggcgcgcgtctggtcggtagtgaaagccaacgcctacggccacggtattgaacgcgtctggagcgcgctgggcgccacagatggtttcgctatgctcaaccttgaagaggcgattaccctgcgtgagcgcgggtggaaagggccgatattgatgctggaggggtttttccatgcgcaagacctggaggcgtatgacacttatcggctgaccacctgcatccacagtaactggcagttgaaagcgctgcaaaatgcgcggcttaacgcgccgctggatatctatgtcaaagtcaacagcggcatgaaccgactcggttttcagcctgagcgggcgcagaccgtctggcagcaattgcgggcaatgcgcaatgtcggtgaaatgaccctgatgtcacattttgctcaggccgatcatccggaaggtatcggggaggcgatgaggcgtattgcgctggcgacggaaggtcttcagtgtgcatactcgttatcaaattcggcagcgacgctgtggcatccccaggcgcattatgactgggtcaggccgggcattattttgtacggcgcgtcgccgtcaggacagtggcgggatattgccgataccggactaaaacctgtgatgacgctgagtagcgaaattattggcgtgcagacgctgagcgcgggtgaaagggtaggctatggcggagggtattctgtgactcaggaacaacgcattggcatcgtcgcggcgggttatgccgatggctatccacgccatgcgccgaccgggacgcctgtgctggtggacggtatccgtaccagaacagtaggcaccgtttcaatggatatgctggcggtggatttgacgccgtgtccgcaggcgggaatcggcacgccggttgaattatggggcaaagaaattaaggtcgatgatgtcgcttctgcggcaggcacgctgggctatgagctactgtgcgccgtagcgccgcgtgtgccgtttgtgacaacgtaa

SEQ ID NO: 20 - protein, 356 aa, Artificial sequence
MTRPIQASLDLQVMKQNLAIVRRAAPEARVWSVVKANAYGHGIERVWSALGATDGFAMLNLEEAITLRERGWKGPILMLEGFFHAQDLEAYDTYRLTTCIHSNWQLKALQNARLNAPLDIYVKVNSGMNRLGFQPERAQTVWQQLRAMRNVGEMTLMSHFAQADHPEGIGEAMRRIALATEGLQCAYSLSNSAATLWHPQAHYDWVRPGIILYGASPSGQWRDIADTGLKPVMTLSSEIIGVQTLSAGERVGYGGGYSVTQEQRIGIVAAGYADGYPRHAPTGTPVLVDGIRTRTVGTVSMDMLAVDLTPCPQAGIGTPVELWGKEIKVDDVASAAGTLGYELLCAVAPRVPFVTT

SEQ ID NO: 21 - DNA, 1080 bp, Artificial sequence
  source 1..1080: mol_type = other DNA
atgcaagcggcaactgttgtgattaaccgccgcgctctgcgacacaacctgcaacgtcttcgtgaactggcccctgccagtaaaatggttgcggtggtgaaagcgaacgcttatggtcacggtcttcttgagaccgcgcgaacgctccccgatgctgacgcctttggcgtagcccgtctcgaagaagctctgcgactgcgtgcggggggaatcaccaaacctgtactgttactcgaaggcttttttgatgccagagatctgccgacgatttctgcgcaacattttcataccgccgtgcataacgaagaacagctggctgcgctggaagaggctagcctggacgagccggttaccgtctggatgaaactcgataccggtatgcaccgtctgggcgtaaggccggaacaggctgaggcgttttatcatcgcctgacccagtgcaaaaacgttcgtcagccggtgaatatcgtcagccattttgcgcgcgcggatgaaccaaaatgtggcgcaaccgagaaacaactcgctatctttaataccttttgcgaaggcaaacctggtcaacgttccattgccgcgtcgggtggcattctgctgtggccacagtcgcattttgactgggtgcgcccgggcatcattctttatggcgtctcgccgctggaagatcgctccaccggtgccgattttggctgtcagccagtgatgtcactaacctccagcctgattgccgtgcgtgagcataaagccggagagcctgttggttatggtggaacctgggtaagcgaacgtgatacccgtcttggcgtagtcgcgatgggctatggcgatggttatccgcgcgccgcgccgtccggtacgccagtgctggtgaacggtcgcgaagtaccgattgtcgggcgcgtggcgatggatatgatctgcgtagacttaggtccacaggcgcaggacaaagccggggatccggtcattttatggggcgaaggtttgcccgtagaacgtatcgctgaaatgacgaaagtaagcgcttacgaacttattacgcgcctgacttcaagggtcgcgatgaaatacgtggattaa

SEQ ID NO: 22 - protein, 359 aa, Artificial sequence
MQAATVVINRRALRHNLQRLRELAPASKMVAVVKANAYGHGLLETARTLPDADAFGVARLEEALRLRAGGITKPVLLLEGFFDARDLPTISAQHFHTAVHNEEQLAALEEASLDEPVTVWMKLDTGMHRLGVRPEQAEAFYHRLTQCKNVRQPVNIVSHFARADEPKCGATEKQLAIFNTFCEGKPGQRSIAASGGILLWPQSHFDWVRPGIILYGVSPLEDRSTGADFGCQPVMSLTSSLIAVREHKAGEPVGYGGTWVSERDTRLGVVAMGYGDGYPRAAPSGTPVLVNGREVPIVGRVAMDMICVDLGPQAQDKAGDPVILWGEGLPVERIAEMTKVSAYELITRLTSRVAMKYVD

SEQ ID NO: 23 - DNA, 1071 bp, Artificial sequence
  source 1..1071: mol_type = other DNA
atgacccgtccgatacaggccagcctcgatctgcaggcattaaaacagaatctgtccattgtccgccaggccgcgacgcacgcgcgcgtctggtcggtggtaaaagcgaacgcttacgggcatggtattgagcgtatctggagcgcgatcggggccaccgatggctttgcattgcttaacctggaagaggcaataacgttacgtgagcgcggctggaaaggaccgatcctgatgctggaaggatttttccatgctcaggatctggagatttatgaccagcaccgcctgaccacctgcgtacacagcaactggcagctcaaagcactgcaaaatgcgcggctaaaagcaccgttggatatttatcttaaagtgaacagtgggatgaatcggttgggcttccagcccgatcgcgtgcttaccgtctggcagcagttgcgggcaatggcgaatgttggcgaaatgaccctgatgtcgcattttgccgaagcggaacatcctgatggaatttccggcgcgatggcgcgtattgagcaggcggcggaggggctggagtgtcggcgttcgttgtccaattcggcggcgactctgtggcacccggaagcgcattttgactgggttcggcctggcattattttgtatggcgcttcgccgtccggtcagtggcgtgatatcgccaataccggattacgtccggtgatgacgctaagcagtgagattattggtgtccagacgctaaaagcgggcgagcgtgtgggctacggcggtcgctatactgcgcgcgatgaacagcgaatcggcattgtcgccgcagggtacgccgacggttatccgcgccacgcgcctaccggtacccctgttttagtggacggcgtgcgcaccatgacggtggggaccgtctcgatggatatgctagcggtcgatttaacgccttgcccgcaggcgggtattggtacgccggttgagctgtggggcaaggagatcaaaattgatgatgtcgccgccgctgccggaacggtgggctatgagttgatgtgcgcgctggcgctacgcgtcccggttgtgacggtgtaa

SEQ ID NO: 24 - protein, 356 aa, Artificial sequence [sequence omitted]

SEQ ID NO: 25 - DNA, 1080 bp, Artificial sequence
  source 1..1080: mol_type = other DNA
atgcaagcggcaactgttgtgattaaccgccgcgctctgcgacacaacctgcaacgtcttcgtgaactggcacctgccagtaaaatggttgcggtggtgaaagcgaacgcttatggtcacggtcttcttgagaccgcgcgaacgctccccgatgctgacgcctttggcgtagcccgtctcgaagaagctctgcgactgcgtgcggggggaatcaccaaacctgtactgttactcgaaggcttttttgatgccagagatctgccgacgatttctgcgcaacattttcataccgccgtgcataacgaagaacagctggctgcgctggaagaggctagcttggacgagccggttaccgtctggatgaaactcgataccggtatgcaccgtctgggcgtaaggccggaacaggctgaggcgttttatcatcgcctgacccagtgcaaaaacgttcgtcagccggtgaatatcgtcagccattttgcgcgcgcggatgaaccaaaatgtggcgcaaccgagaaacaactcgctatctttaataccttttgcgaaggcaaacctggtcaacgttccattgccgcgtcgggtggcattctgctgtggccacagtcgcattttgactgggtgcgcccgggcatcattctttatggcgtctcgccgctggaagatcgctccaccggtgccgattttggctgtcagccagtgatgtcactaacctccagcctgattgccgtgcgtgagcataaagccggagagcctgttggttatggtggaacctgggtaagcgaacgtgatacccgtcttggcgtagtcgcgatgggctatggcgatggttatccgcgcgccgcgccgtccggtacgccagtgctggtgaacggtcgcgaagtaccgattgtcgggcgcgtggcgatggatatgatctgcgtagacttaggtccacaggcgcaggacaaagccggggatccggtcattttatggggcgaaggtttgcccgtagaacgtatcgctgaaatgacgaaagtaagcgcttacgaacttattacgcgcctgacttcaagggtcgcgatgaaatacgtggattaa

SEQ ID NO: 26 - protein, 359 aa, Artificial sequence; identical to SEQ ID NO: 22

SEQ ID NO: 27 - DNA, 1071 bp, Artificial sequence
  source 1..1071: mol_type = other DNA
atgacccgtccgatacaggccagcctcgatctgcaggcattaaaacagaatctgtccattgtccgccaggccgcgccgcacgcgcgcgtctggtcggtggtaaaagcgaacgcttacgggcatggtattgagcgtatctggagcgcgctcggggccaccgatggctttgcattacttaacctggaagaggcaataacgttacgtgagcgcggctggaaggggccgatcctgatgctggaaggatttttccatgctcaggatctggagatttatgaccagcaccgcctgaccacctgcgtacacagcaactggcagctcaaagcactgcaaaatgcgcggctaaaagcaccgttggatatttatcttaaagtgaacagtgggatgaatcggttgggcttccagtccgatcgcgtgcttaccgtctggcagcagttgcgggcaatggcgaatgttggcgaaatgaccctgatgtcgcattttgctgaagcggaacatcctgatggaatttccggcgcgatggcgcgtattgagcaggcggcggaggggctggagtgtcggcgttcgttgtccaattcggcggcgactctgtggcacccggaagcgcattttgactgggttcggcctggcattattttgtatggcgcttcgccgtccggtcagtggcgtgatatcgccaataccggattacgtccggtgatgacgctaagcagtgagattattggtgtccagacgctaaaagcgggcgagcgtgtgggctacggcggtcgctatactgcgcgcgatgaacagcgaatcggcattgtcgccgcaggatacgccgacggttatccgcgccatgcgcctaccggtgctcctgttttagtggacggcgtgcgcaccatgacggtggggaccgtctcgatggatatgctggcggttgatttaacgccttgcccgcaggcggggattggtacgccggttgagctgtggggcaaggagatcaaaattgatgatgtcgccgccgctgccggaacggtgggctatgagttgatgtgcgcactggcgttacgcgtcccggttgtgacagtgtaa

SEQ ID NO: 28 - protein, 356 aa, Artificial sequence
MTRPIQASLDLQALKQNLSIVRQAAPHARVWSVVKANAYGHGIERIWSALGATDGFALLNLEEAITLRERGWKGPILMLEGFFHAQDLEIYDQHRLTTCVHSNWQLKALQNARLKAPLDIYLKVNSGMNRLGFQSDRVLTVWQQLRAMANVGEMTLMSHFAEAEHPDGISGAMARIEQAAEGLECRRSLSNSAATLWHPEAHFDWVRPGIILYGASPSGQWRDIANTGLRPVMTLSSEIIGVQTLKAGERVGYGGRYTARDEQRIGIVAAGYADGYPRHAPTGAPVLVDGVRTMTVGTVSMDMLAVDLTPCPQAGIGTPVELWGKEIKIDDVAAAAGTVGYELMCALALRVPVVTV

SEQ ID NO: 29 - DNA, 1080 bp, Artificial sequence
  source 1..1080: mol_type = other DNA
atgcaagcggcaactgtagtcattaaccgccgcgctctgcgacacaacctgcaacgtctgcgtgaactggcgcccgccagcaaactagttgcggtggtgaaagcgaacgcctacggacacggtcttcttgagaccgcgcgaacgctccctgacgccgatgcttttggcgtcgcccgtcttgaagaagctctgcgcctgcgcgcgggcggtatcggccagccgattctgctgctggaggggttctttgaggctgccgacctggcggtgatttccgcccagcgcctgcacacggcggtacacagcccggaacagctggcggcgctggaggaagcggatttacccgagccggtcaccgtatggatgaagctggataccggaatgcatcgattaggcgttctgcctgagcaggccgaagcgttttatcagcgtcttagccagtgtaaaaacgtccgccagccggtcaacgtggtcagccattttgcccgtgcggatgagcctgagtgcggcgcgaccgaacgtcagctggatatctttaccaccttcacggaagggaaaccgggactgcgctctatcgccgcatccggcggtatattgctgtggccccagtcgcatttcgactgggcgcgtccggggatcattctctacggcgtgtcgccgctcgacggtagctctaccggcgcggactttggctgccagccggtgatgtctctgacctcgagcctgattgcggtccgcgagcataaagccggggagccggtgggctacggcggaacctggatcagcgagcgtgatacgcgtttaggggtggtggcgatgggctacggtgacggctatccgcgcgctgcgccgtccgggaccccggtgctggtcaacggccgcgaagtgccgattgtgggtcgcgtggcgatggatatgatttgcgtcgatctcgggcccgaagcgcaggataaatcgggcgacccggtggtgctgtggggcgaaggcctgcccgtcgagcgtattgccgaaatcacaaaagtaagtgcttacgaacttattacccgcctgacttcacgggtatcaatgaagtacgtggattga

SEQ ID NO: 30 - protein, 359 aa, Artificial sequence
MQAATVVINRRALRHNLQRLRELAPASKLVAVVKANAYGHGLLETARTLPDADAFGVARLEEALRLRAGGIGQPILLLEGFFEAADLAVISAQRLHTAVHSPEQLAALEEADLPEPVTVWMKLDTGMHRLGVLPEQAEAFYQRLSQCKNVRQPVNVVSHFARADEPECGATERQLDIFTTFTEGKPGLRSIAASGGILLWPQSHFDWARPGIILYGVSPLDGSSTGADFGCQPVMSLTSSLIAVREHKAGEPVGYGGTWISERDTRLGVVAMGYGDGYPRAAPSGTPVLVNGREVPIVGRVAMDMICVDLGPEAQDKSGDPVVLWGEGLPVERIAEITKVSAYELITRLTSRVSMKYVD

SEQ ID NO: 31 - DNA, 1071 bp, Artificial sequence
  source 1..1071: mol_type = other DNA
atgtctcgtcctgtaaaggccagcattgatatgtcagccttacgccagaatcagcacattgttcgtcgcgcggcacccggttcgcgcctgtgggcggtggtcaaagccaatgcttatggccacggtctggcgagggtctggaacgcgcttagcgccgcggacggtttcgcgatgctgaatcttgaagaggcgatcctgctgcgcgagctgggctggaaagggccaatactgatgctggaaggctttttccacgccgatgagctggccctgtttgataagtaccgtttgaccaccagcgtgcacagtaactggcaaatcaaggcgctgcagcaggcgaagctgcacgcgccgctcgatatctacgtcaaggtgaatagcgggatgaatcggctggggtttatgccggatcgtctgcacgtcgtctggcagcagctgcgagcgctgcataacgtcagtgaaatgacgttaatgtcacattttgccgaagcggaaaacccggacggcatcgtggagccgatgcggcgtattgagcaggcggcggaaggactggattgcccgcgctcgctggcgaattcggcggccaccctgtggcatccggagtcgcattttaactgggtgaggccggggatcgtgctgtacggcgcttcgccttccggcctgtggcaggatgtggccaacaccgggctgaagccggtgatgacgctaagcagcgaaattattgccgtacagaacctgaaagccggtgaagcggtcggctacggcgcaacctggcgtacggcggaggagcggcgcatcggcatcgttgcctgcggctacgccgatggctacccgcgtctggcgccaagcggtacgccggtgctggttgacggcgttcgcaccgcgacggtagggcgcatctcgatggatatgctggcagtggatttgactccctgcccgcaggcagggatcggtgccccggtcgagctgtggggcaaagagattaaaatcgacgatgtcgcatccgcctgcggcaccgtcgggtatgagttaatgtgcgcgctggcgccgcgcgtaccggttgtgacggtgtaa

SEQ ID NO: 32 - protein, 356 aa, Artificial sequence
MSRPVKASIDMSALRQNQHIVRRAAPGSRLWAVVKANAYGHGLARVWNALSAADGFAMLNLEEAILLRELGWKGPILMLEGFFHADELALFDKYRLTTSVHSNWQIKALQQAKLHAPLDIYVKVNSGMNRLGFMPDRLHVVWQQLRALHNVSEMTLMSHFAEAENPDGIVEPMRRIEQAAEGLDCPRSLANSAATLWHPESHFNWVRPGIVLYGASPSGLWQDVANTGLKPVMTLSSEIIAVQNLKAGEAVGYGATWRTAEERRIGIVACGYADGYPRLAPSGTPVLVDGVRTATVGRISMDMLAVDLTPCPQAGIGAPVELWGKEIKIDDVASACGTVGYELMCALAPRVPVVTV

SEQ ID NO: 33 - DNA, 1080 bp, Artificial sequence
  source 1..1080: mol_type = other DNA
atgaaagcggcaacagcagtaatcgaccgccgcgctctgcgacataatttgcaacaggtacggcgcatggcgccgcaaagtcgcctgattgctgttgtgaaagcaaacgcttatggccatgggttattagagatagcacatactttgcaggatgcagattgctacggtgtagcgcggatcggtgaagcactgatgctccgatctggtgggatcgtgaaaccgattttgttgttggaagggttctttgcagcagaagatctgccggttctggtggccaaccgcattgaaacagcagtacatagtattgagcagttggaagcattggaagctgccgagctttctgcgccaatcaatgtctggatgaaactcgataccggtatgcaccgtctgggcgttcgcccggaacaagctgaggctttttaccagcgcttaagtgcgtgtaacaatgttattcagccagtcaatatcatgagccattttagccgtgctgatgagccacaagtggataccacccgccagcaactggactgttttgatactttcgccgccgataagcctggcaagcaatctattgcggcatctggtggcatattactgtggccagaagcgcaccgtgattgggttcgtccgggaatcatcttgtacggtgtttcgccgatggatgagccttatgccagtcattttggtctattacctgcaatggcattgaaatccagtctgattgctgtgcgtgagcacaaagccggtgagcctgtgggttatggtggcacttgggtgagtgagcgtgatacccgtctgggtgtggtggcgatcggttatggagacggttatccgcgtagcgctccttcaggcaccccgatgtggttgaatggccgcgaagttggcattgtgggccgggtttcaatggatatgatttctgttgatctcgggccaaatgcaaaagataaagtgggtgacgaagtattgctgtggggggctgaactgccggttgaaaaaattgcagcgtgcacaggtatcagcgcctacgaattgattacaaagctgacctcccgcgtcgcgatggaatatttaggtgaataa

SEQ ID NO: 34 - protein, 359 aa, Artificial sequence
MKAATAVIDRRALRHNLQQVRRMAPQSRLIAVVKANAYGHGLLEIAHTLQDADCYGVARIGEALMLRSGGIVKPILLLEGFFAAEDLPVLVANRIETAVHSIEQLEALEAAELSAPINVWMKLDTGMHRLGVRPEQAEAFYQRLSACNNVIQPVNIMSHFSRADEPQVDTTRQQLDCFDTFAADKPGKQSIAASGGILLWPEAHRDWVRPGIILYGVSPMDEPYASHFGLLPAMALKSSLIAVREHKAGEPVGYGGTWVSERDTRLGVVAIGYGDGYPRSAPSGTPMWLNGREVGIVGRVSMDMISVDLGPNAKDKVGDEVLLWGAELPVEKIAACTGISAYELITKLTSRVAMEYLGE

SEQ ID NO: 35 - DNA, 1068 bp, Artificial sequence
  source 1..1068: mol_type = other DNA
atgcctcgcccgatatctgccacgctgaatttatctgcgctgcaccataatctgaatgttgcgcgcagtcatgtgggaacagcaaaaatttggtcagtggtgaaagccaatgcctacggtcatggtttagcgcgtgtctggcaagggctggcggcgacggatggatttgctttactggatttaaacgaagctatcctgctgcgagaacagggctggcaagggccaattttattgctggagggtttctttcaagcgcaggatttggtgctgctggatcattatcgcttgacgacggcggtgcacagtgactggcaacttgaggctatcaaagcggcccgcctgacggctccactcaatatttacttgaagtttaatagcggtatgaatcgtttagggtttccaattggtcaggcggaagctgtgtggcaatgggccaacagcctcagcaatgtcggcgaaatcacattaatgagccactttgctaatgcagataatcctattggtgctgatgagcaatttgctcagatccagcaggccagtgggcatattccggcggcccgctgttttgccaattcagcggcgattttgcgcaacccacaaactcattatgactgggtgcgcccagggattattctctacggcgcatcccccagtggtgatattgcagatattgccggtcttggtttgcgcccggtgatgagtttgcacagtgagattatcgcgctgcaatcattatccgccggtcaaagtgtgggttatggtagccgttatcgcgccaccggtgcgcagcgcataggagtggtcgcttgtggttatgccgatggttatccgcgtgtcgcaccaacgggaacacctatcatggtggatggtatattgacgcacacaatgggggcgatttcgatggatatgctcaccgtggatctcacgccatgtccgcaagcgcagatgggcagcaaagtcgaaatatggggtgagaatgtgcccattgacaatgtggcacaggccgcgggaacggtggggtatgagttgatgtgtgcgctggcagccagggttacccttctgacttga

SEQ ID NO: 36 - protein, 355 aa, Artificial sequence
MPRPISATLNLSALHHNLNVARSHVGTAKIWSVVKANAYGHGLARVWQGLAATDGFALLDLNEAILLREQGWQGPILLLEGFFQAQDLVLLDHYRLTTAVHSDWQLEAIKAARLTAPLNIYLKFNSGMNRLGFPIGQAEAVWQWANSLSNVGEITLMSHFANADNPIGADEQFAQIQQASGHIPAARCFANSAAILRNPQTHYDWVRPGIILYGASPSGDIADIAGLGLRPVMSLHSEIIALQSLSAGQSVGYGSRYRATGAQRIGVVACGYADGYPRVAPTGTPIMVDGILTHTMGAISMDMLTVDLTPCPQAQMGSKVEIWGENVPIDNVAQAAGTVGYELMCALAARVTLLT

SEQ ID NO: 37 - DNA, 1083 bp, Artificial sequence
  source 1..1083: mol_type = other DNA
atgaacgtaaaaccggcgacagcgaaaattagttcgcacgccttaaaacagaatttagaaataattaaacaaaaagcaccaaatagcaaaattattgctgtggttaaagcaaacgcctatggtcacggcgttgtattcgttgcttcaaccttagaacaaaatgttgattgctttggcgtggcgcgtttagaagaggctttagcattacgctccaacggcattactaaaccgattttattgcttgaaggttttttcaatgaacaagatttgcctattctagccgttaataatattgaaaccgtggtacacaatcacgaacagcttgatgctttaaaacgtgcgaatttaccaagtccaattaaagtttggttaaaaatagatacgggaatgcatcgcttgggcgttgctcttgatgaagtggattatttttatcaagaactgaaaaaactccctcaaattcaaccgcacttaggctttgtcagccatttcagccgagccgatgaactagaatcagattacactcagctccaaatcaatcgttttttatccgccacaaaagataaacaaggtgaacgcactatcgcagcttctggcggcattcttttctggcctgaatctcatctggaatgtatccgcccaggcattattatgtacggcatttctccaactgatactatcggtaaagagtttggcttaacgccagtgatgaatttaacctcgtcattaattgccgttcgccatcataaacaaggcgatcctgtaggttacggcggtatttggacaagtccacgagatactaaaattggcgtggtcgcaatgggttatggcgatggttatccgcgcgatgtgccagaaggtacacctgtttatttaaatggccgtcttgtaccaattgttggacgtgtgtcaatggatatgcttactgttgatttaggcgcagatagccaagatttggtaggcgatgaagtaattttatggggcaaggaattacctattgaaaccgtagctaaattcacaggcattttaagctacgagctaattacaaaattaacacctcgtgttataactgaatacgttgattaa

SEQ ID NO: 38 - protein, 360 aa, Artificial sequence
MNVKPATAKISSHALKQNLEIIKQKAPNSKIIAVVKANAYGHGVVFVASTLEQNVDCFGVARLEEALALRSNGITKPILLLEGFFNEQDLPILAVNNIETVVHNHEQLDALKRANLPSPIKVWLKIDTGMHRLGVALDEVDYFYQELKKLPQIQPHLGFVSHFSRADELESDYTQLQINRFLSATKDKQGERTIAASGGILFWPESHLECIRPGIIMYGISPTDTIGKEFGLTPVMNLTSSLIAVRHHKQGDPVGYGGIWTSPRDTKIGVVAMGYGDGYPRDVPEGTPVYLNGRLVPIVGRVSMDMLTVDLGADSQDLVGDEVILWGKELPIETVAKFTGILSYELITKLTPRVITEYVD

SEQ ID NO: 39 - DNA, 1077 bp, Artificial sequence
  source 1..1077: mol_type = other DNA
atgcgtcccctcgttgccaccgtcgacctttccgccattcgccacaactatgccctggccaagcgctgcgcgccgcagcgccaggcgttcgcggtggtcaaggcgaacgcctatggccacggtgcgcgcgaagtggttaccgcgttgcacgacgatgccgatggcttcgccgtggcctgcctggaggaggccgcggaagtccgcgccttgcacgccagcgcgcgcatcctgttgctggaaggctgcttcgaggcgagcgaatacgccctcgccgggcaattgcgcctggacctggtgatccagggcgcggaacagggcgaggcgttcctcgccgccggcctggatattccactcaacgtctggctcaagctcgactccggcatgcaccgcctgggcttcgatcctgccgcgctgcgcgcctggcatgcgcgcctgcgcagccatcccggtgtgcgcgagctgaacctgatcagccatttcgcctgcgccgacgaacgcaaccatccgctcaccgaacagcagctggagagtttcctcggcctgctcgacctggacttcgaccagcgcagcctggccaattcggcggcggtgctgactatcccggccgcccacatggactggctgcggccgggaatcatgctctacgggtcgaccccgctggccgacctcagtgctgccgaactgggcctgaagccggccatgagcctgggcgcgcagttgatttcactgcgcgaggtggccgtgggtgagagcgtcggctacggcgccacctggatcgccgagcggccggcgcggatcggcacggtcagttgcggctacgccgacggctatccgcgtaccgcgccagccgggactccggtactggtcgggggacgccgcgcgatcctggccgggcgggtctcgatggacatgctggcggtcgacctctccgacctgccggaggctcgcgttggcgacccggtggagttgtggggcgccgggttgtcggtggacgaggtcgcccgtgcctgcggcacccttggctacgagcttctgagcaaggtcacggctcgggttccgcgacgctacagccactga

SEQ ID NO: 40 - protein, 358 aa, Artificial sequence
MRPLVATVDLSAIRHNYALAKRCAPQRQAFAVVKANAYGHGAREVVTALHDDADGFAVACLEEAAEVRALHASARILLLEGCFEASEYALAGQLRLDLVIQGAEQGEAFLAAGLDIPLNVWLKLDSGMHRLGFDPAALRAWHARLRSHPGVRELNLISHFACADERNHPLTEQQLESFLGLLDLDFDQRSLANSAAVLTIPAAHMDWLRPGIMLYGSTPLADLSAAELGLKPAMSLGAQLISLREVAVGESVGYGATWIAERPARIGTVSCGYADGYPRTAPAGTPVLVGGRRAILAGRVSMDMLAVDLSDLPEARVGDPVELWGAGLSVDEVARACGTLGYELLSKVTARVPRRYSH

SEQ ID NO: 41 - DNA, 1074 bp, Artificial sequence
  source 1..1074: mol_type = other DNA
atgcgccccgcccgtgccctgatcgacctgcaagcccttcgtcacaactatcggctggcccgcgaggccaccggcgcccgtgcgctcgcggtgatcaaggcggacgcatacggccacggcgcggtgcgctgtgccgaagcgctggcggccgaggccgatggcttcgccgtggcctgcatcgaggagggcctggagctgcgcgaggccggtatccgccagccgatcctgctgctggagggcttcttcgaggcgtccgagctggagctgatcgtcgcccacgacttctggtgcgtggtgcattgcgcctggcaattggaggcgatcgaacgcgccagcctggcccgcccgctgaacgtctggctgaagatggattcgggcatgcaccgcgtcggcttcttccccgaggacttcagcgccgcccacgagcgcctgcgggccagcggcaaggtggcgaagatcgtgatgatgagtcacttctcccgcgccgacgaactggattgcccgcgcaccgaggaacagctcgccgccttcgcggccgcgagccagggcctggaaggcgagatcagcctgcgcaattcgccagccgtgctcggctggccgaaggtgcccagcgattgggtacgtccgggcatcctgctctacggagccacgccgttcgagcgcgcacatccgctggccgaccgcttgcgcccggtgatgaccctagaatcgaaggtgatcagcgtccgcgacctgccggccggcgaaccggtcggctacggcgcgcgctacagcaccgagcgtagccagcgcatcggcgtggtcgccatgggctacgccgatggctatccgcgccacgccgccgacggcacccttgtgttcatcgacggcaagccggggcgcctggttggccgggtatcgatggacatgctcaccgtcgaccttaccgaccatccccaggccgggctgggcagccgggtcgaactatggggcccgaacgtgccggtcggcgccctggcggcgcagttcggcagcattccctaccagctgctgtgcaacctgaaaagggtgccgcgcgtctattccggggcttga

SEQ ID NO: 42 - protein, 357 aa, Artificial sequence
MRPARALIDLQALRHNYRLAREATGARALAVIKADAYGHGAVRCAEALAAEADGFAVACIEEGLELREAGIRQPILLLEGFFEASELELIVAHDFWCVVHCAWQLEAIERASLARPLNVWLKMDSGMHRVGFFPEDFSAAHERLRASGKVAKIVMMSHFSRADELDCPRTEEQLAAFAAASQGLEGEISLRNSPAVLGWPKVPSDWVRPGILLYGATPFERAHPLADRLRPVMTLESKVISVRDLPAGEPVGYGARYSTERSQRIGVVAMGYADGYPRHAADGTLVFIDGKPGRLVGRVSMDMLTVDLTDHPQAGLGSRVELWGPNVPVGALAAQFGSIPYQLLCNLKRVPRVYSGA

SEQ ID NO: 43 - DNA, 1147 bp, Artificial sequence
  source 1..1147: mol_type = other DNA
gcggccgcgactagtgaacctcttcgagggacctaataacttcgtatagcatacattatacgaagttatattaagggttccggatcctaagcttgatatctaagggcaccaataactgccttaaaaaaattacgccccgccctgccactcatcgcagtactgttgtaattcattaagcattctgccgacatggaagccatcacagacggcatgatgaacctgaatcgccagcggcatcagcaccttgtcgccttgcgtataatatttgcccatggtgaaaacgggggcgaagaagttgtccatattggccacgtttaaatcaaaactggtgaaactcacccagggattggctgagacgaaaaacatattctcaataaaccctttagggaaataggccaggttttcaccgtaacacgccacatcttgcgaatatatgtgtagaaactgccggaaatcgtcgtggtattcactccagagcgatgaaaacgtttcagtttgctcatggaaaacggtgtaacaagggtgaacactatcccatatcaccagctcaccgtctttcattgccatacggaattccggatgagcattcatcaggcgggcaagaatgtgaataaaggccggataaaacttgtgcttatttttctttacggtctttaaaaaggccgtaatatccagctgaacggtctggttataggtacattgagcaactgactgaaatgcctcaaaatgttctttacgatgccattgggatatatcaacggtggtatatccagtgatttttttctccattttagcttccttagctcctgaaaatctcgataactcaaaaaatacgcccggtagtgatcttatttcattatggtgaaagttggaacctcttacgtgccgatcaacgtctcattttcgccaaaagttggcccagggcttcccggtatcaacagggacaccaggatttatttattctgcgaagtgatcttccgtcacaggtatttattcggcgcaaagtgcgtcgggtgatgctgccgatatcggtacccgggatcctaagcttggctggacgtaaactcctcttcagacctaataacttcgtatagcatacattatacgaagttatattaagggttattgaatatgatcgggcggccgc

SEQ ID NO: 44 - DNA, 237 bp, Artificial sequence
  source 1..237: mol_type = other DNA
gtaaacgcaacggatggctgaccgctgcggggtttgtggttaaccaccttaatcactcttaatgagggcggtcattctacggcaaaccaccgtgatcgccaatccttgttgcgaattactgacttagctttatagtcagaaagcgtgtcaaagtgaaatattcttgtttgcagggataaaagtgacctgacgcaatatttgtcttttcttgcttattaataatgttgtcacgaaaag

SEQ ID NO: 45 - DNA, 1107 bp, Artificial sequence
  source 1..1107: mol_type = other DNA
atgaaaaatgttggttttatcggctggcgcggaatggtcggctctgttctcatgcaacgcatggtagaggagcgcgatttcgacgctattcgccctgttttcttttctacctcccagtttggacaggcggcgcccaccttcggcgacacctccaccggcacgctacaggacgcttttgatctggatgcgctaaaagcgctcgatatcatcgtgacctgccagggcggcgattataccaacgaaatttatccaaagctgcgcgaaagcggatggcagggttactggattgatgcggcttctacgctgcgcatgaaagatgatgccattattattctcgacccggtcaaccaggacgtgattaccgacggcctgaacaatggcgtgaagacctttgtgggcggtaactgtaccgttagcctgatgttgatgtcgctgggcggtctctttgcccataatctcgttgactgggtatccgtcgcgacctatcaggccgcctccggcggcggcgcgcgccatatgcgcgagctgttaacccagatgggtcagttgtatggccatgtcgccgatgaactggcgacgccgtcttccgcaattcttgatattgaacgcaaagttacggcattgacccgcagcggcgagctgccggttgataactttggcgtaccgctggcgggaagcctgatcccctggatcgacaaacagctcgataacggccagagccgcgaagagtggaaaggccaggcggaaaccaacaagattctcaatactgcctctgtgattccggttgatggtttgtgtgtgcgcgtcggcgcgctgcgctgtcacagccaggcgttcaccatcaagctgaaaaaagaggtatccattccgacggtggaagaactgctggcggcacataatccgtgggcgaaagtggtgccgaacgatcgtgatatcactatgcgcgaattaaccccggcggcggtgaccggcacgttgactacgccggttggtcgtctgcgtaagctgaacatggggccagagttcttgtcggcgtttaccgtaggcgaccagttgttatggggcgccgccgagccgctgcgtcgaatgctgcgccagttggcgtag

SEQ ID NO: 46 - protein, 368 aa, Artificial sequence
MKNVGFIGWRGMVGSVLMQRMVEERDFDAIRPVFFSTSQFGQAAPTFGDTSTGTLQDAFDLDALKALDIIVTCQGGDYTNEIYPKLRESGWQGYWIDAASTLRMKDDAIIILDPVNQDVITDGLNNGVKTFVGGNCTVSLMLMSLGGLFAHNLVDWVSVATYQAASGGGARHMRELLTQMGQLYGHVADELATPSSAILDIERKVTALTRSGELPVDNFGVPLAGSLIPWIDKQLDNGQSREEWKGQAETNKILNTASVIPVDGLCVRVGALRCHSQAFTIKLKKEVSIPTVEELLAAHNPWAKVVPNDRDITMRELTPAAVTGTLTTPVGRLRKLNMGPEFLSAFTVGDQLLWGAAEPLRRMLRQLA

SEQ ID NO: 47 - DNA, 60 bp, Artificial sequence
  source 1..60: mol_type = other DNA
acgaaaagtacggcattgataatcattttcaatatcatttaattaactataatgaaccaa

SEQ ID NO: 48 - DNA, 238 bp, Artificial sequence
  source 1..238: mol_type = other DNA
cacaatacgggaacgcagtttatccaacacgagttttactccctgtttcaacaatcatcctattttgccatatcagaaaaataacatagcggtataaatcaacaattccatatgaaattgctgctaccaccaatacaactttaactgccttaaatcaaaaattgtcgcagcaaggttaactaaaatcccagttcgttaacatttttgcgttttgatagcgcaaccttcaggaaaaatt

SEQ ID NO: 49 - DNA, 208 bp, Artificial sequence
  source 1..208: mol_type = other DNA
gagttttactccctgtttcaacaatcatcctattttgccatatcagaaaaataacatagcggtataaatcaacaattccatatgaaattgctgctaccaccaatacaactttaactgccttaaatcaaaaattgtcgcagcaaggttaactaaaatcccagttcgttaacatttttgcgttttgatagcgcaaccttcaggaaaaatt

SEQ ID NO: 50 - DNA, 315 bp, Artificial sequence
  source 1..315: mol_type = other DNA
aggcggtgactccttgtaatcctgaataaaatgatagcactgaataaaatgacaatgccaagtaccgctattctgccacattgctaacctatgaaaatgggctatatcgacaaattttgcatcagaacatcttcagatgtattgctaaatatcagaagagtgtcaccaatgcgaaagaaactgccttaaatcaaggtgcgatgtgaagaggttaactaaaattgccgctcgataaaataccaagatcatctatgccctcacatctgcaacttgaatctgcaacttgaagtatggggggtatatcagggaaattct

SEQ ID NO: 51 - DNA, 451 bp, Artificial sequence
  source 1..451: mol_type = other DNA
gagctttactccctgatagctatagtcctgctattttgccatatccgaagcacaacatagcggcgtaaatcaacaaactgtcgtcagttgtacctcattattggtgccatcaatacgccattagctgccttaaatcaaaaattgtcgcgtatgggttaattaaaatcccagctcgttaacaaatttgcgatcgactacatcaggataaattatggagctgctctgcccagccggaaatcttccggcgcttaaggcggccatcgaaaatggggccgatgcggtctatatcgggctgaaagatgataccaacgcccgccattttgctggcctcaactttacggagaaaaagcttcaggaagccgttaccttcgtccaccagcaccgccgcaaactgcatatcgccatcaataccttcgcccatcctgatggctacgcccgctggcaacgcgcg

SEQ ID NO: 52 - DNA, 248 bp, Artificial sequence
  source 1..248: mol_type = other DNA
gggcttttctccttgccagatcacaatggccgttattgtgccatatcggccaggcgagatagcggctcaaatcaagctttgcgccttcgcaggtacccctttatagatgccatcaatacgacattagctgccttaaatcaaaaattgtcgcggacgggttaactaaaatcgccgttcgttaacaatttcgctgcctttatgcagcgcgccaggccgcatacggcctgcttttattttcaggacacgct

SEQ ID NO: 53 - DNA, 221 bp, Artificial sequence
  source 1..221: mol_type = other DNA
aagctttactccatgaatgcaatagttccgctattgtgccatatcacataaacaacatagcggcgtaaatcaacaaaaacgcgatgacggccgccagttattggcgccgccaatacacttttaactgcctcaaatcaaaaattgtcaccagaaggttaactaaaatccctgctcgttaaccattcagcgtccctgacgggccgcatttttcaggaaaaatt

SEQ ID NO: 54 - DNA, 154 bp, Artificial sequence
  source 1..154: mol_type = other DNA
tcccgcctcctttgagatcaataaaacctatcgtaagcgggttaaaaaaaagccaggctatctcatcaatgaccgtttcactgccctaaatcaacatttacccaaagcgccatgactagactcgtgctccatctgcatcacgagaggattgagt

SEQ ID NO: 55 - DNA, 154 bp, Artificial sequence; identical to SEQ ID NO: 54
  source 1..154: mol_type = other DNA

SEQ ID NO: 56 - DNA, 258 bp, Artificial sequence
  source 1..258: mol_type = other DNA
gtactttactccctgaaatagataatcctcgatattgtgccacagacatggtgccgccagctggctcaaaatcaacaattggcgaacttaacggcacggggtcatcctgtgcttttcagagtaccaatacgccattagctgccccaaatcaaaaattgccatcaactggttaattaaaatcgcggttcgttaacaattacgctggcctgccaggtcatggtacagcacgggcgcctgcccggataaccaggaaaaatt

SEQ ID NO: 57 - DNA, 144 bp, Artificial sequence
  source 1..144: mol_type = other DNA
catcagaacctcttattaattccgcaaaagattgagctacctcaagcccctacgcggcagcatcccctagaatttttccgaaagacttcttcgccgccggtgcggcgatacattgttaacggggcattctggggcattttattc

SEQ ID NO: 58 - DNA, 124 bp, Artificial sequence
  source 1..124: mol_type = other DNA
cattttttaactgttctaccaaaatttgcgctatctcaatttgggccaggaaagcataacttagactttcaaggttaattattttcctagtttatatttgtgaagcataacggtggagttagtg

SEQ ID NO: 59 - DNA, 130 bp, Artificial sequence
  source 1..130: mol_type = other DNA
ctcttttccgcagatgtacgaaaaattgcgctatctcaagctgggtagcgcacgcatcccgtagacttcccccactgaattttttctctggtttatattttcgaagcatacccaagaggtggaatgagtc

SEQ ID NO: 60 - DNA, 3650 bp, Artificial sequence
  source 1..3650: mol_type = other DNA
gaattctcagccaaacgtctcttcaggccactgactagcgataactttccccacaacggaacaactctcattgcatgggatcattgggtactgtgggtttagtggttgtaaaaacacctgaccgctatccctgatcagtttcttgaaggtaaactcatcacccccaagtctggctatgcagaaatcacctggctcaacagcctgctcagggtcaacgagaattaacattccgtcaggaaagcttggcttggagcctgttggtgcggtcatggaattaccttcaacctcaagccagaatgcagaatcactggcttttttggttgtgcttacccatctctccgcatcacctttggtaaaggttctaagcttaggtgagaacatccctgcctgaacatgagaaaaaacagggtactcatactcacttctaagtgacggctgcatactaaccgcttcatacatctcgtagatttctctggcgattgaagggctaaattcttcaacgctaactttgagaatttttgtaagcaatgcggcgttataagcatttaatgcattgatgccattaaataaagcaccaacgcctgactgccccatccccatcttgtctgcgacagattcctgggataagccaagttcatttttctttttttcataaattgctttaaggcgacgtgcgtcctcaagctgctcttgtgttaatggtttcttttttgtgctcatacgttaaatctatcaccgcaagggataaatatctaacaccgtgcgtgttgactattttacctctggcggtgataatggttgcatgtactaaggaggttgcgcatgcaggtaccaatgtccaatttactgaccgtacaccaaaatttgcctgcattaccggtcgatgcaacgagtgatgaggttcgcaagaacctgatggacatgttcagggatcgccaggcgttttctgagcatacctggaaaatgcttctgtccgtttgccggtcgtgggcggcatggtgcaagttgaataaccggaaatggtttcccgcagaacctgaagatgttcgcgattatcttctatatcttcaggcgcgcggtctggcagtaaaaactatccagcaacatttgggccagctaaacatgcttcatcgtcggtccgggctgccacgaccaagtgacagcaatgctgtttcactggttatgcggcggatccgaaaagaaaacgttgatgccggtgaacgtgcaaaacaggctctagcgttcgaacgcactgatttcgaccaggttcgttcactcatggaaaatagcgatcgctgccaggatatacgtaatctggcatttctggggattgcttataacaccctgttacgtatagccgaaattgccaggatcagggttaaagatatctcacgtactgacggtgggagaatgttaatccatattggcagaacgaaaacgctggttagcaccgcaggtgtagagaaggcacttagcctgggggtaactaaactggtcgagcgatggatttccgtctctggtgtagctgatgatccgaataactacctgttttgccgggtcagaaaaaatggtgttgccgcgccatctgccaccagccagctatcaactcgcgccctggaagggatttttgaagcaactcatcgattgatttacggcgctaaggatgactctggtcagagatacctggcctggtctggacacagtgcccgtgtcggagccgcgcgagatatggcccgcgctggagtttcaataccggagatcatgcaagctggtggctggaccaatgtaaatattgtcatgaactatatccgtaacctggatagtgaaacaggggcaatggtgcgcctgctggaagatggcgattaggggtaccgagctcatgaacgcttattacattcaggatcgtcttgaggctcagagctgggcgcgtcactaccagcagctcgcccgtgaagagaaagaggcagaactggcagacgacatggaaaaaggcctgccccagcacctgtttgaatcgctatgcatcgatcatttgcaacgccacggggccagcaaaaaatccattacccgtgcgtttgatgacgatgttgagtttcaggagcgcatggcagaacacatccggtacatggttgaaaccattgctcaccaccaggttgatattgattcagaggtataaaacgaatgagtactgcactcgcaacgctggctgggaagctggctgaacgtgtcggcatggattctgtcgacccacaggaactgatcaccactcttcgccagacggcatttaaaggtgatgccagcgatgcgcagttcatcgcattactgatcgttgccaaccagtacggccttaatccgtggacgaaagaaatttacgcctttcctgataagcagaatggcatcgttccggtggtgggcgttgatggctggtcccgcatcatcaatgaaaaccagcagtttgatggcatggactttgagcaggacaatgaatcctgtacatgccggatttaccgcaaggaccgtaatcatccgatctgcgttaccgaatggatggatgaatgccgccgcgaaccattcaaaactcgcgaaggcagagaaatcacggggccgtggcagtcgcatcccaaacggatgttacgtcataaagccatgattcagtgtgcccgtctggccttcggatttgctggtatctatgacaaggatgaagccgagcgcattgtcgaaaatactgcatacactgcagaacgtcagccggaacgcgacatcactccggttaacgatgaaaccatgcaggagattaacactctgctgatcgccctggataaaacatgggatgacgacttattgccgctctgttcccagatatttcgccgcgacattcgtgcatcgtcagaactgacacaggccgaagcagtaaaagctcttggattcctgaaacagaaagccgcagagcagaaggtggcagcatgacaccggacattatcctgcagcgtaccgggatcgatgtgagagctgtcgaacagggggatgatgcgtggcacaaattacggctcggcgtcatcaccgcttcagaagttcacaacgtgatagcaaaaccccgctccggaaagaagtggcctgacatgaaaatgtcctacttccacaccctgcttgctgaggtttgcaccggtgtggctccggaagttaacgctaaagcactggcctggggaaaacagtacgagaacgacgccagaaccctgtttgagttcacttccggcgtgaatgttactgaatccccgatcatctatcgcgacgaaagtatgcgtaccgcctgctctcccgatggtttatgcagtgacggcaacggccttgaactgaaatgcccgtttacctcccgggatttcatgaagttccggctcggtggtttcgaggccataaagtcagcttacatggcccaggtgcagtacagcatgtgggtgacgcgaaaaaatgcctggtactttgccaactatgacccgcgtatgaagcgtgaaggcctgcattatgtcgtgattgagcgggatgaaaagtacatggcgagttttgacgagatcgtgccggagttcatcgaaaaaatggacgaggcactggctgaaattggttttgtatttggggagcaatggcgatgactcgag

SEQ ID NO: 61 - DNA, 1133 bp, Artificial sequence
  source 1..1133: mol_type = other DNA
actagtgaacctcttcgagggacctaataacttcgtatagcatacattatacgaagttatattaagggttccggatcctaattgatatctaagggcaccaataactgccttaaaaaaattatgcaccaccttgccattcatcacaatactgttgcagttcattcagcatacgaccaacatgaaaaccatcacaaactgcatgatgaacctgaattgccagcggcatcagaactttatcaccctgggtgtaatatttgcccatcgtaaaaaccggtgcgaaaaagttatccatattggccacattcagatcaaatgaggtaaagctaacccacggatttgcgctaacaaagaacatgttttcgataaagcctttcggaaaatatgccaggttttcaccataacatgcaacatcctggctatagatgtgcaggaactgacgaaaatcatcatgatattctgaccacaggctgctaaaggtttcggtctgttcatgaaaaacggtataacacggatgaacgctatcccaaataaccagttcaccatctttcattgccatacgaaattccggatgggcattcatcagacgtgccagaatatgaataaaggcagggtagaacttgtgtttgttctttttcacggttttcagaaatgcggttatatccagctgaacggtctgattataggtacactgtgcaacgctctgaaatgcttcaaagtgttctttacgatgccactggctaatatcaacggtggtataaccggtgattttcttttccattttagcttccttagctcctgaaaatctcgataactcaaaaaatacgcccggtagtgatcttatttcattatggtgaaagttggaacctcttacgtgccgatcaacgtctcattttcgccaaaagttggcccagggcttcccggtatcaacagggacaccaggatttatttattctgcgaagtgatcttccgtcacaggtatttattcggcgcaaagtgcgtcgggtgatgctgccgatatcggacccgggatcctaattggctggacgtaaactcctcttcagacctaataacttcgtatagcatacattatacgaagttatattaagggttattgaatatgatcgggcggccgc

SEQ ID NO: 62 - DNA, 216 bp, Artificial sequence
  source 1..216: mol_type = other DNA
tgcccggacggcataatattacgacgctgacctggcggactgctgccgtcaggtcaatatgctaaaaatcccttcatttctaataaccctataattaatcaacgaaattataatgtttctaaaattagaatataatttataaacattatttaaatgttgttacttaagtgttaccgttgatgccgcgcaaatctcacctgcaataaagcgactaaa

SEQ ID NO: 63 - DNA, 71 bp, Artificial sequence
  source 1..71: mol_type = other DNA
atggaatccctgacgttacaacccatcgcgcgggtcgatggcgccattaaccgatcatattcaataaccct

SEQ ID NO: 64 - DNA, 72 bp, Artificial sequence
  source 1..72: mol_type = other DNA
gaagacttaggcaggcgtactcattcgcgccagttgttcgaaataatcaggactagtgaacctcttcgaggg

SEQ ID NO: 65 - DNA, 20 bp, Artificial sequence
  source 1..20: mol_type = other DNA
cggacaatacgctggacaag

SEQ ID NO: 66 - DNA, 20 bp, Artificial sequence
  source 1..20: mol_type = other DNA
gcggctttgtaggttgacat

SEQ ID NO: 67 - DNA, 22 bp, Artificial sequence
  source 1..22: mol_type = other DNA
tccttagctcctgaaaatctcg

SEQ ID NO: 68 - DNA, 20 bp, Artificial sequence
  source 1..20: mol_type = other DNA
tgtggcgtgttacggtgaaa

SEQ ID NO: 69 - DNA, 29 bp, Artificial sequence
  source 1..29: mol_type = other DNA
aaactgcagtgcccggacggcataatatt

SEQ ID NO: 70 - DNA, 33 bp, Artificial sequence
  source 1..33: mol_type = other DNA
ccgctcgagtttagtcgctttattgcaggtgag

SEQ ID NO: 71 - DNA, 37 bp, Artificial sequence
  source 1..37: mol_type = other DNA
atttgcggccgcgtaaacgcaacggatggctgaccgc

SEQ ID NO: 72 - DNA, 35 bp, Artificial sequence
  source 1..35: mol_type = other DNA
cccaagcttcttttcgtgacaacattattaataag

SEQ ID NO: 73 - DNA, 50 bp, Artificial sequence
  source 1..50: mol_type = other DNA
cccaagctttggagcgaaaccgatgaaaaatgttggttttatcggctggc

SEQ ID NO: 74 - DNA, 34 bp, Artificial sequence
  source 1..34: mol_type = other DNA
ccgctcgagctacgccaactggcgcagcattcga

SEQ ID NO: 75 - DNA, 62 bp, Artificial sequence
  source 1..62: mol_type = other DNA
gacgaaaagtacggcattgataatcattttcaatatcatttaattaactataatgaaccaac

SEQ ID NO: 76 - DNA, 70 bp, Artificial sequence
  source 1..70: mol_type = other DNA
tcgagttggttcattatagttaattaaatgatattgaaaatgattatcaatgccgtacttttcgtctgca

SEQ ID NO: 77 - DNA, 60 bp, Artificial sequence
  source 1..60: mol_type = other DNA
cgcatacacagcacatctctttgcaggaaaaaaacgctgaacctcttcgagggacctaat

SEQ ID NO: 78 - DNA, 61 bp, Artificial sequence
  source 1..61: mol_type = other DNA
gaaccacacgcaggcccgataagcgctgcaatagccaacgaaaagtacggcattgataatc

SEQ ID NO: 79 - DNA, 37 bp, Artificial sequence
  source 1..37: mol_type = other DNA
atttgcggccgcgcgtgaacgcagtttatctaacacg

SEQ ID NO: 80 - DNA, 35 bp, Artificial sequence
  source 1..35: mol_type = other DNA
cccaagcttttatcctgagggttacgtctgagacg

SEQ ID NO: 81 - DNA, 32 bp, Artificial sequence
  source 1..32: mol_type = other DNA
atttgcggccgccgctgcactggtaaaagacg

SEQ ID NO: 82 - DNA, 30 bp, Artificial sequence
  source 1..30: mol_type = other DNA
cccaagcttaactccaccgttatgcttcac

SEQ ID NO: 83 - DNA, 38 bp, Artificial sequence
  source 1..38: mol_type = other DNA
atttgcggccgcctcttcataaaacccgtcagtgtaag

SEQ ID NO: 84 - DNA, 32 bp, Artificial sequence
  source 1..32: mol_type = other DNA
cccaagcttctgaaataacattgtgaacggca

SEQ ID NO: 85 - DNA, 37 bp, Artificial sequence
  source 1..37: mol_type = other DNA
atttgcggccgctcattaaatttaactcaaattttgc

SEQ ID NO: 86 - DNA, 35 bp, Artificial sequence
  source 1..35: mol_type = other DNA
cccaagcttgacctacgttaattacctcattgacg

SEQ ID NO: 87 - DNA, 33 bp, Artificial sequence
  source 1..33: mol_type = other DNA
atttgcggccgccgtaacgctaaaaccaacacc

SEQ ID NO: 88 - DNA, 30 bp, Artificial sequence
  source 1..30: mol_type = other DNA
cccaagcttccctcctcaaaaaaagcctag

SEQ ID NO: 89 - DNA, 34 bp, Artificial sequence
  source 1..34: mol_type = other DNA
atttgcggccgcagacgcgatgtataacggctct

SEQ ID NO: 90 - DNA, 32 bp, Artificial sequence
  source 1..32: mol_type = other DNA
cccaagcttcactaactccaccgttatgcttc

SEQ ID NO: 91 - DNA, 33 bp, Artificial sequence
  source 1..33: mol_type = other DNA
atttgcggccgcgttaatattggcggggtggat

SEQ ID NO: 92 - DNA, 30 bp, Artificial sequence
  source 1..30: mol_type = other DNA
cccaagcttgactccttgctcatcgcatga

SEQ ID NO: 93 - DNA, 32 bp, Artificial sequence
  source 1..32: mol_type = other DNA
atttgcggccgcaaagcagcattctgggcaaa

SEQ ID NO: 94 - DNA, 34 bp, Artificial sequence
  source 1..34: mol_type = other DNA
cccaagcttaactctctctttattaagtcggcga

SEQ ID NO: 95 - DNA, 43 bp, Artificial sequence
  source 1..43: mol_type = other DNA
cccaagctttggagcgaaaccgatgcaagcggcaacagtcgtc

SEQ ID NO: 96 - DNA, 38 bp, Artificial sequence
  source 1..38: mol_type = other DNA
ccgctcgagttaatcaatatacttcatcgccacccttg

SEQ ID NO: 97 - DNA, 42 bp, Artificial sequence
  source 1..42: mol_type = other DNA
cccaagctttggagcgaaaccgatgcaagcggcaactgttgt

SEQ ID NO: 98 - DNA, 31 bp, Artificial sequence
  source 1..31: mol_type = other DNA
ccgctcgagttaatccacgtatttcatcgcg

SEQ ID NO: 99 - DNA, 42 bp, Artificial sequence
  source 1..42: mol_type = other DNA
cccaagctttggagcgaaaccgatgacccgccctatacaggc

SEQ ID NO: 100 - DNA, 30 bp, Artificial sequence
  source 1..30: mol_type = other DNA
cccaagcttttacgttgtcacaaacggcac

SEQ ID NO: 101 - DNA, 42 bp, Artificial sequence
  source 1..42: mol_type = other DNA
cccaagctttggagcgaaaccgatgacccgtccgatacaggc

SEQ ID NO: 102 - DNA, 29 bp, Artificial sequence
  source 1..29: mol_type = other DNA
cccaagcttttacaccgtcacaaccggga

SEQ ID NO: 103 - DNA, 35 bp, Artificial sequence
  source 1..35: mol_type = other DNA
ccgctcgagattggttctgtgttaccaagttctgc

SEQ ID NO: 104 - DNA, 35 bp, Artificial sequence
  source 1..35: mol_type = other DNA
aaaactgcagaacattatttgccgttgtaataacg

SEQ ID NO: 105 - DNA, 34 bp, Artificial sequence
  source 1..34: mol_type = other DNA
ccgctcgagatctgagggttggcttccttgtaag

SEQ ID NO: 106 - DNA, 35 bp, Artificial sequence
  source 1..35: mol_type = other DNA
aaaactgcagccgacatgtccgatagcattattgc

SEQ ID NO: 107 - DNA, 32 bp, Artificial sequence
  source 1..32: mol_type = other DNA
ccgctcgagtgcaggtctcctgagaaccacac

SEQ ID NO: 108 - DNA, 34 bp, Artificial sequence
  source 1..34: mol_type = other DNA
aaaactgcagtgaagtaacaacactcccgacatc

SEQ ID NO: 109 - DNA, 30 bp, Artificial sequence
  source 1..30: mol_type = other DNA
ccgctcgagacatacccctcaagtggcgtc

SEQ ID NO: 110 - DNA, 32 bp, Artificial sequence
  source 1..32: mol_type = other DNA
aaaactgcagtagcgttgtctgtttagcgtgc

SEQ ID NO: 111 - DNA, 32 bp, Artificial sequence
  source 1..32: mol_type = other DNA
ccgctcgagaagcgatgttaaaaacagagccg

SEQ ID NO: 112 - DNA, 36 bp, Artificial sequence
  source 1..36: mol_type = other DNA
aaaactgcagaatgtcatgcctccagtgaatgttac

SEQ ID NO: 113 - DNA, 29 bp, Artificial sequence
  source 1..29: mol_type = other DNA
ccgctcgagccgcgatctccatagtgact

SEQ ID NO: 114 - DNA, 29 bp, Artificial sequence
  source 1..29: mol_type = other DNA
aaactgcagtgtttttaggcggataaggc

SEQ ID NO: 115 - DNA, 29 bp, Artificial sequence
  source 1..29: mol_type = other DNA
ccgctcgagtgcaggtctcctggagtcca

SEQ ID NO: 116 - DNA, 36 bp, Artificial sequence
  source 1..36: mol_type = other DNA
aaactgcaggaacacagtatctacagggtgattctg

SEQ ID NO: 117 - DNA, 31 bp, Artificial sequence
  source 1..31: mol_type = other DNA
ccgctcgagaagcgatgttaaaaacgaagcg

SEQ ID NO: 118 - DNA, 29 bp, Artificial sequence
  source 1..29: mol_type = other DNA
aaactgcagctgacattgcctgcgaaaac

SEQ ID NO: 119 - DNA, 20 bp, Artificial sequence
  source 1..20: mol_type = other DNA
ggtacgcaagattggggtac

SEQ ID NO: 120 - DNA, 20 bp, Artificial sequence
  source 1..20: mol_type = other DNA
gaaaacgctcgcctgttctt

SEQ ID NO: 121 - DNA, 20 bp, Artificial sequence
  source 1..20: mol_type = other DNA
tgtcagctctttacccagcg

SEQ ID NO: 122 - DNA, 71 bp, Artificial sequence
  source 1..71: mol_type = other DNA
gcaatacgatgatgagtaactctccgtcattcttttaacaaggaattcaaccgatcatattcaataaccct

SEQ ID NO: 123 - DNA, 72 bp, Artificial sequence
  source 1..72: mol_type = other DNA
tgcgcgatacaagccggataagcgcaagcgccacccggcccgccgcgtatgactagtgaacctcttcgaggg

SEQ ID NO: 124 - DNA, 20 bp, Artificial sequence
  source 1..20: mol_type = other DNA
caggtcttacgccgacagaa

SEQ ID NO: 125 - DNA, 20 bp, Artificial sequence
  source 1..20: mol_type = other DNA
gttgctgaagaaccgggtga

SEQ ID NO: 126 - DNA, 20 bp, Artificial sequence
  source 1..20: mol_type = other DNA
cgacggcgatgcttaaaggc

SEQ ID NO: 127 - DNA, 20 bp, Artificial sequence
  source 1..20: mol_type = other DNA
taaagttctgatgccgctgg

SEQ ID NO: 128 - DNA, 20 bp, Artificial sequence
  source 1..20: mol_type = other DNA
cggtggtcttatggggtgaa

SEQ ID NO: 129 - DNA, 67 bp, Artificial sequence
  source 1..67: mol_type = other DNA
cacccccccgcaacgtttgcatagcgcgcataactgataaaggaagtgaacaggaaacagctatgac

SEQ ID NO: 130 - DNA, 67 bp, Artificial sequence
  source 1..67: mol_type = other DNA
acgtcgacccgcccccaagtggaccggtcgacgccttagcctgaattagggtaaaacgacggccagt

SEQ ID NO: 131 - DNA, 32 bp, Artificial sequence
  source 1..32: mol_type = other DNA
atttgcggccgccacaatacgggaacgcagtt

SEQ ID NO: 132 - DNA, 30 bp, Artificial sequence
  source 1..30: mol_type = other DNA
cccaagcttaatttttcctgaaggttgcgc

SEQ ID NO: 133 - DNA, 20 bp, Artificial sequence
  source 1..20: mol_type = other DNA
aaacccgccagcttacactg

SEQ ID NO: 134 - DNA, 70 bp, Artificial sequence
  source 1..70: mol_type = other DNA
gcaatacgatgatgagtaactctccgtcattcttttaacaaggaattcaagaacaggaaacagctatgac

SEQ ID NO: 135 - DNA, 67 bp, Artificial sequence
  source 1..67: mol_type = other DNA
tgcgcgatacaagccggataagcgcaagcgccacccggcccgccgcgtatgtaaaacgacggccagt

SEQ ID NO: 136 - DNA, 20 bp, Artificial sequence
  source 1..20: mol_type = other DNA
gcaccttaggctggacgatg

SEQ ID NO: 137 - DNA, 20 bp, Artificial sequence
  source 1..20: mol_type = other DNA
cgacgcagagtttcaggatt

SEQ ID NO: 138 - DNA, 72 bp, Artificial sequence
  source 1..72: mol_type = other DNA
cacccccccgcaacgtttgcatagcgcgcataactgataaaggaagtgaagaacctcttcgagggacctaat

SEQ ID NO: 139 - DNA, 74 bp, Artificial sequence
  source 1..74: mol_type = other DNA
acgtcgacccgcccccaagtggaccggtcgacgccttagcctgaattaggacgaaaagtacggcattgataatc

SEQ ID NO: 140 - DNA, 20 bp, Artificial sequence
  source 1..20: mol_type = other DNA
tcgccactggactttctgct

SEQ ID NO: 141 - DNA, 20 bp, Artificial sequence
  source 1..20: mol_type = other DNA
ctgcgtcgtcctaccttcag

SEQ ID NO: 142 - DNA, 20 bp, Artificial sequence
  source 1..20: mol_type = other DNA
aagaggtatccattccgacg

SEQ ID NO: 143 - DNA, 20 bp, Artificial sequence
  source 1..20: mol_type = other DNA
aagggagcatcaggcgaata

SEQ ID NO: 144 - DNA, 20 bp, Artificial sequence
  source 1..20: mol_type = other DNA
aactgcgttcccgtattgtg

SEQ ID NO: 145 - DNA, 20 bp, Artificial sequence
  source 1..20: mol_type = other DNA
taaccgctccctggaacaac

SEQ ID NO: 146 - DNA, 20 bp, Artificial sequence
  source 1..20: mol_type = other DNA
ggtaagcaacgtaacggtcc